European Patent Application EP 4 582 561 A1, published July 9, 2025. Title: Combination of Differentially Methylated Regions, Kit, and Use thereof. Applicant: BGI GENOMICS CO., LTD. Application WO PCT/CN2022/116795, filed September 2, 2022. The sequence listing filed with the application follows.

SEQUENCE LISTING (212 sequences)

SEQ ID NO: 1 - DNA, 1297 bp, Homo sapiens
  source 1..1297: mol_type = genomic DNA
cgccgtagctgcgtccccagaaccgggagacttaaggcatctttattgcgggatcctcacacggcctcctgggcccggcgatactcatagacgctgccgtgctcgggaaaggccagtgcttgcgggggcgaccccggcggtggggcggggtcctccgggtccccatagccaccgccgccgggcgtgtggagacagaacacatcctgttggcgcgggggggggcggggaggcgggctcagtgcaggcgtggcccctccctgtcacctgcgcagtcccctccccaccgggcagcgtccatcacccgcccccatggaccacggaggcccggtacgcgccccctttccttccggggccaaattaaactcggcctctggtcaggtctgcaactgttccccctctgtgggatggggccgggaggggaggggaggggagggggacaggacaggccgcggcccttaccccggggtacacggtcaccgacgtcttgccgcccagattcaccgtccggccgtttttgcggatcagcaggtttaggccgcgggcgccaggctcgccccctgcggagggaggcgaggagtccagagagaccaggggcgggggtgggggcgggggcggggagggccgcgagggctggggaaccgcgcaccgtggagcccgtatggccggaaggcgcggcgctcggtcagcactgacagcagcgcctcctcacgaaagagcagctcgcgggtgacgccgtcgccgcctcggaagcggcctctgccccccgagccccccgccgcagctcgaagcggcgcaggatgaccgggtacctgcgagggcgaggacgagggcaaagactcagcgtggcccgagccccggctcccacccggccgtgcccccagcctccgcgcacgccgctcaccggctctccaggatctcagggtcggtgatgcgtgtgttggtcatgtggctgtgcacaccgctgcgcccgtgccagctgggacccgcgcccgcgccgcccgccaccgtctcgtagtagcccatgtgggcgttgcccagggtcacgttgttcatgcagccctggtgagggcacctggtcgctgcgctgggctggggcagggcgtccccacctcgccctcccgctcctactccagcctgcccacccagtccgcccccgagctgcgcccaccccgcccccgcacctgggaggcggcgcaggccccaaaggcccccaggatgacatccaccacgcgctgcgacgtgagcacgttgccgcccaccaccgccgcctcgggcgacgggtccaggatggagcctc

SEQ ID NO: 2 - DNA, 1366 bp, Homo sapiens
  source 1..1366: mol_type = genomic DNA
agtctaatcatggcaagttttaactattgatgtaagagttttaactattgattttgctttcatcaaaagcaaagccattcacacagtatttaacaaaaaccctcgggctctgctaggttcttgtttactgttaaaacagtttaaaggcagggtcttgatcacttaaaatactcttagaagggaaagtaacattttaaaggattaacagtggaaaaagaatatccctgttcctcttccttcccccaagtcctcaacatgtgaaaaatagagttgataagtaaggagatttaaggcagaacccgaggcctacggagcagttaccttctacggcaatttcaagggtggatggtgcgagcgccgctggggcagctggcgttctggttcttactccgtgggaaaatggccctgagcccgactggcttgaggcttagacaggtgaccccgcgaagcgggtgggcaggcgcggccgaggggcgggaggcgggcagcctccgtgattggccggcggagggggcggtgtagcgacccgaggagggaagaggactccaagcgccatggccgctgccgcccgagcccgggtcgcgtacttgctgaggcaactgcaacgcgcagcgtgagtgcggggccggcgggcgggcaggggaccgcagggtgcccacgcagccccctgggtgtgacccgctcagatcctgcgcagtcttctccgcttactttcaagaattcggagaatttggataccgccctgggctcccaccgcgcgccaggcggaacagcgaggtcacagagtgcgcgatgcagcctctcagggcgcagtgaggcagcctttactctgcttgtctaccgttaaagaaactgaggcccagagaggacctggtcccacatcgtagcaggcagtggagagcttggcacggtggccaagacaaattcatgtatgcaattgacacatatttattgggcatatattatgtgccaaaaactattctaggttctggggatacaaagatgaaaggctctggagcagtttgaggtctagtggggaatgggatgaggggacgaggctaaaaccggctatagcagactgggtgtagaagggaaggatggatgtgagaagtcgcagagtcacacttcctggcatgtacagggagtcagggtattcaatgtcatgacacgcctgcctcccagcagaaatgtgaggtacatcctggtcacctgataaatacttgctgactgtgcaagtgcacaagtctgcctgggaaacatggaaaagtttgagctcacaggtgcagatcagtaggaggaaaggcgagggactggcgaggaacgtcaggcagagagaagagcaacaccagcgatggagatgcagtcc

SEQ ID NO: 3 - DNA, 20 bp, synthetic construct
  source 1..20: mol_type = other DNA
gaattaggcgtcgtagttgc

SEQ ID NO: 4 - DNA, 20 bp, synthetic construct
  source 1..20: mol_type = other DNA
cgcaaacactaacctttccc

SEQ ID NO: 5 - DNA, 22 bp, synthetic construct
  source 1..22: mol_type = other DNA
gggttcggcgatatttatagac

SEQ ID NO: 6 - DNA, 16 bp, synthetic construct
  source 1..16: mol_type = other DNA
ccccaccgccgaaatc

SEQ ID NO: 7 - DNA, 24 bp, synthetic construct
  source 1..24: mol_type = other DNA
agtacggtagcgtttatgagtatc

SEQ ID NO: 8 - DNA, 20 bp, synthetic construct
  source 1..20: mol_type = other DNA
aactaaacgccgtaactacg

SEQ ID NO: 9 - DNA, 20 bp, synthetic construct
  source 1..20: mol_type = other DNA
ttatcgtcggggtcgttttc

SEQ ID NO: 10 - DNA, 26 bp, synthetic construct
  source 1..26: mol_type = other DNA
acatctttattacgaaatcctcacac

SEQ ID NO: 11 - DNA, 19 bp, synthetic construct
  source 1..19: mol_type = other DNA
tcgtcgggtttaggaggtc

SEQ ID NO: 12 - DNA, 21 bp, synthetic construct
  source 1..21: mol_type = other DNA
actcgaaacacgaactaaacg

SEQ ID NO: 13 - DNA, 25 bp, synthetic construct
  source 1..25: mol_type = other DNA
tatttttattgcgggatttttatac

SEQ ID NO: 14 - DNA, 25 bp, synthetic construct
  source 1..25: mol_type = other DNA
caaaatatattctatctccacacgc

SEQ ID NO: 15 - DNA, 22 bp, synthetic construct
  source 1..22: mol_type = other DNA
cgtagttgcgtttttagaatcg

SEQ ID NO: 16 - DNA, 22 bp, synthetic construct
  source 1..22: mol_type = other DNA
tataaaaacccgaaaaaccccg

SEQ ID NO: 17 - DNA, 21 bp, synthetic construct
  source 1..21: mol_type = other DNA
gggtagtgcgtttgtagtttc

SEQ ID NO: 18 - DNA, 22 bp, synthetic construct
  source 1..22: mol_type = other DNA
cgacaacgtctataaatatcgc

SEQ ID NO: 19 - DNA, 24 bp, synthetic construct
  source 1..24: mol_type = other DNA
ttttggaggggtttacggattatc

SEQ ID NO: 20 - DNA, 24 bp, synthetic construct
  source 1..24: mol_type = other DNA
ccaaaaaaccgtataaaaatcccg

SEQ ID NO: 21 - DNA, 23 bp, synthetic construct
  source 1..23: mol_type = other DNA
aaggtaagtatagatgaggggcg

SEQ ID NO: 22 - DNA, 21 bp, synthetic construct
  source 1..21: mol_type = other DNA
cgcaaacactaacctttcccg

SEQ ID NO: 23 - DNA, 20 bp, synthetic construct
  source 1..20: mol_type = other DNA
gaggtcgtgtgaggatttcg

SEQ ID NO: 24 - DNA, 21 bp, synthetic construct
  source 1..21: mol_type = other DNA
aacaatacgcctacaactccg

SEQ ID NO: 25 - DNA, 22 bp, synthetic construct
  source 1..22: mol_type = other DNA
gggtagtgcgtttgtagtttcg

SEQ ID NO: 26 - DNA, 25 bp, synthetic construct
  source 1..25: mol_type = other DNA
acacgacaacgtctataaatatcgc

SEQ ID NO: 27 - DNA, 23 bp, synthetic construct
  source 1..23: mol_type = other DNA
tcgggtagtgcgtttgtagtttc

SEQ ID NO: 28 - DNA, 24 bp, synthetic construct
  source 1..24: mol_type = other DNA
ggtttacggattatcgggtagtgc

SEQ ID NO: 29 - DNA, 24 bp, synthetic construct
  source 1..24: mol_type = other DNA
cgacaacgtctataaatatcgccg

SEQ ID NO: 30 - DNA, 19 bp, synthetic construct
  source 1..19: mol_type = other DNA
gggcgttgtttagggttac

SEQ ID NO: 31 - DNA, 18 bp, synthetic construct
  source 1..18: mol_type = other DNA
aaacgcaactcgaaaacg

SEQ ID NO: 32 - DNA, 17 bp, synthetic construct
  source 1..17: mol_type = other DNA
ccctaccccaacccaac

SEQ ID NO: 33 - DNA, 21 bp, synthetic construct
  source 1..21: mol_type = other DNA
cgttcgtgttagttgggattc

SEQ ID NO: 34 - DNA, 25 bp, synthetic construct
  source 1..25: mol_type = other DNA
cataaacaacgtaaccctaaacaac

SEQ ID NO: 35 - DNA, 23 bp, synthetic construct
  source 1..23: mol_type = other DNA
gggacgttttgttttagtttagc

SEQ ID NO: 36 - DNA, 19 bp, synthetic construct
  source 1..19: mol_type = other DNA
cccgtaccaactaaaaccc

SEQ ID NO: 37 - DNA, 19 bp, synthetic construct
  source 1..19: mol_type = other DNA
tatttgcgagggcgaggac

SEQ ID NO: 38 - DNA, 22 bp, synthetic construct
  source 1..22: mol_type = other DNA
cctaaaaaaccgataaacgacg

SEQ ID NO: 39 - DNA, 21 bp, synthetic construct
  source 1..21: mol_type = other DNA
cgttcgtgttagttgggatgc

SEQ ID NO: 40 - DNA, 24 bp, synthetic construct
  source 1..24: mol_type = other DNA
taaacaacgtaaccctaaacaccg

SEQ ID NO: 41 - DNA, 19 bp, synthetic construct
  source 1..19: mol_type = other DNA
gggcgttgtttagggttgc

SEQ ID NO: 42 - DNA, 17 bp, synthetic construct
  source 1..17: mol_type = other DNA
cctaccccaacccaccg

SEQ ID NO: 43 - DNA, 21 bp, synthetic construct
  source 1..21: mol_type = other DNA
cgttcgtgttagttgggcttc

SEQ ID NO: 44 - DNA, 24 bp, synthetic construct
  source 1..24: mol_type = other DNA
taaacaacgtaaccctaaaccacg

SEQ ID NO: 45 - DNA, 21 bp, synthetic construct
  source 1..21: mol_type = other DNA
cgttcgtgttagttgggatcc

SEQ ID NO: 46 - DNA, 21 bp, synthetic construct
  source 1..21: mol_type = other DNA
cgttcgtgttagttggggttc

SEQ ID NO: 47 - DNA, 24 bp, synthetic construct
  source 1..24: mol_type = other DNA
taaacaacgtaaccctaaacgacg

SEQ ID NO: 48 - DNA, 24 bp, synthetic construct
  source 1..24: mol_type = other DNA
taaacaacgtaaccctaaacaacg

SEQ ID NO: 49 - DNA, 17 bp, synthetic construct
  source 1..17: mol_type = other DNA
cctaccccaacccaacg

SEQ ID NO: 50 - DNA, 18 bp, synthetic construct
  source 1..18: mol_type = other DNA
aagcggcgtaggatgatc

SEQ ID NO: 51 - DNA, 17 bp, synthetic construct
  source 1..17: mol_type = other DNA
ccgaaactcgaaccacg

SEQ ID NO: 52 - DNA, 19 bp, synthetic construct
  source 1..19: mol_type = other DNA
aaaccgaaactcgaaccac

SEQ ID NO: 53 - DNA, 19 bp, synthetic construct
  source 1..19: mol_type = other DNA
tttaaaacctacgccgcct

SEQ ID NO: 54 - DNA, 21 bp, synthetic construct
  source 1..21: mol_type = other DNA
acgaaataaaaacgccctacc

SEQ ID NO: 55 - DNA, 28 bp, synthetic construct
  source 1..28: mol_type = other DNA
actcgaaaacgaactaaataaacaaact

SEQ ID NO: 56 - DNA, 24 bp, synthetic construct
  source 1..24: mol_type = other DNA
tgaataacgtgattttgggtaacg

SEQ ID NO: 57 - DNA, 24 bp, synthetic construct
  source 1..24: mol_type = other DNA
cgactctccaaaatctcaaaatcg

SEQ ID NO: 58 - DNA, 22 bp, synthetic construct
  source 1..22: mol_type = other DNA
gggtaaagatttagcgtggttc

SEQ ID NO: 59 - DNA, 19 bp, synthetic construct
  source 1..19: mol_type = other DNA
acgaaataaacgcaactcg

SEQ ID NO: 60 - DNA, 19 bp, synthetic construct
  source 1..19: mol_type = other DNA
cgcaactcgaaaacgaact

SEQ ID NO: 61 - DNA, 20 bp, synthetic construct
  source 1..20: mol_type = other DNA
aggatgatcgggtatttgcg

SEQ ID NO: 62 - DNA, 21 bp, synthetic construct
  source 1..21: mol_type = other DNA
caaccacataaccaacacacg

SEQ ID NO: 63 - DNA, 19 bp, synthetic construct
  source 1..19: mol_type = other DNA
gcgaatcccaactaacacg

SEQ ID NO: 64 - DNA, 21 bp, synthetic construct
  source 1..21: mol_type = other DNA
gacgagggtaaagatttagcg

SEQ ID NO: 65 - DNA, 22 bp, synthetic construct
  source 1..22: mol_type = other DNA
ggtaaagatttagcgtggttcg

SEQ ID NO: 66 - DNA, 25 bp, synthetic construct
  source 1..25: mol_type = other DNA
tcggttttttaggattttagggtcg

SEQ ID NO: 67 - DNA, 25 bp, synthetic construct
  source 1..25: mol_type = other DNA
cctcaccaaaactacataaacaacg

SEQ ID NO: 68 - DNA, 29 bp, synthetic construct
  source 1..29: mol_type = other DNA
ttgtatgaataacgtgattttgggtaacg

SEQ ID NO: 69 - DNA, 27 bp, synthetic construct
  source 1..27: mol_type = other DNA
caccgactctccaaaatctcaaaatcg

SEQ ID NO: 70 - DNA, 28 bp, synthetic construct
  source 1..28: mol_type = other DNA
ttatcgattttgagattttggagagtcg

SEQ ID NO: 71 - DNA, 23 bp, synthetic construct
  source 1..23: mol_type = other DNA
ctcgatcaacactaacaacaacg

SEQ ID NO: 72 - DNA, 23 bp, synthetic construct
  source 1..23: mol_type = other DNA
gcgtaggatgatcgggtatttgc

SEQ ID NO: 73 - DNA, 22 bp, synthetic construct
  source 1..22: mol_type = other DNA
cgaatcccaactaacacgaacg

SEQ ID NO: 74 - DNA, 16 bp, synthetic construct
  source 1..16: mol_type = other DNA
tttgcggagggaggcg

SEQ ID NO: 75 - DNA, 18 bp, synthetic construct
  source 1..18: mol_type = other DNA
gcgattccccaaccctcg

SEQ ID NO: 76 - DNA, 23 bp, synthetic construct
  source 1..23: mol_type = other DNA
ggagtttagagagattaggggcg

SEQ ID NO: 77 - DNA, 19 bp, synthetic construct
  source 1..19: mol_type = other DNA
cgaccatacgaactccacg

SEQ ID NO: 78 - DNA, 20 bp, synthetic construct
  source 1..20: mol_type = other DNA
tcgtggagttcgtatggtcg

SEQ ID NO: 79 - DNA, 19 bp, synthetic construct
  source 1..19: mol_type = other DNA
cccgcgaactactctttcg

SEQ ID NO: 80 - DNA, 17 bp, synthetic construct
  source 1..17: mol_type = other DNA
tcgttggggtagttggc

SEQ ID NO: 81 - DNA, 24 bp, synthetic construct
  source 1..24: mol_type = other DNA
cctatctaaacctcaaaccaatcg

SEQ ID NO: 82 - DNA, 20 bp, synthetic construct
  source 1..20: mol_type = other DNA
gttttgggtttttatcgcgc

SEQ ID NO: 83 - DNA, 21 bp, synthetic construct
  source 1..21: mol_type = other DNA
gccctaaaaaactacatcgcg

SEQ ID NO: 84 - DNA, 22 bp, synthetic construct
  source 1..22: mol_type = other DNA
aggtttagataggtgatttcgc

SEQ ID NO: 85 - DNA, 16 bp, synthetic construct
  source 1..16: mol_type = other DNA
aaactacccgcctccc

SEQ ID NO: 86 - DNA, 22 bp, synthetic construct
  source 1..22: mol_type = other DNA
ttggcgttttggtttttatttc

SEQ ID NO: 87 - DNA, 26 bp, synthetic construct
  source 1..26: mol_type = other DNA
gatttaaggtagaattcgaggtttac

SEQ ID NO: 88 - DNA, 21 bp, synthetic construct
  source 1..21: mol_type = other DNA
cacgaaataaaaaccaaaacg

SEQ ID NO: 89 - DNA, 22 bp, synthetic construct
  source 1..22: mol_type = other DNA
cgtagttttttgggtgtgattc

SEQ ID NO: 90 - DNA, 22 bp, synthetic construct
  source 1..22: mol_type = other DNA
aaaacgatatccaaattctccg

SEQ ID NO: 91 - DNA, 24 bp, synthetic construct
  source 1..24: mol_type = other DNA
cgtattttgtgatttcgttgtttc

SEQ ID NO: 92 - DNA, 25 bp, synthetic construct
  source 1..25: mol_type = other DNA
aaaaattcgaaaaatttaaataccg

SEQ ID NO: 93 - DNA, 20 bp, synthetic construct
  source 1..20: mol_type = other DNA
cgtttgtttattcgtttcgc

SEQ ID NO: 94 - DNA, 20 bp, synthetic construct
  source 1..20: mol_type = other DNA
cgccgctaaaacaactaacg

SEQ ID NO: 95 - DNA, 21 bp, synthetic construct
  source 1..21: mol_type = other DNA
cgttttgagaggttgtatcgc

SEQ ID NO: 96 - DNA, 25 bp, synthetic construct
  source 1..25: mol_type = other DNA
gtttagggcggtatttaaatttttc

SEQ ID NO: 97 - DNA, 23 bp, synthetic construct
  source 1..23: mol_type = other DNA
atataacccgctcaaatcctacg

SEQ ID NO: 98 - DNA, 23 bp, synthetic construct
  source 1..23: mol_type = other DNA
tgtatcgcgtattttgtgatttc

SEQ ID NO: 99 - DNA, 21 bp, synthetic construct
  source 1..21: mol_type = other DNA
ccgcttactttcaaaaattcg

SEQ ID NO: 100 - DNA, 23 bp, synthetic construct
  source 1..23: mol_type = other DNA
ggtaattttaagggtggatggtg

SEQ ID NO: 101 - DNA, 23 bp, synthetic construct
  source 1..23: mol_type = other DNA
tcacctatctaaacctcaaacca

SEQ ID NO: 102 - DNA, 29 bp, synthetic construct
  source 1..29: mol_type = other DNA
ggggttatttgtttaagttttaagttagt

SEQ ID NO: 103 - DNA, 27 bp, synthetic construct
  source 1..27: mol_type = other DNA
aaacaattaccttctacracaatttca

SEQ ID NO: 104 - DNA, 25 bp, synthetic construct
  source 1..25: mol_type = other DNA
aagtaaggagatttaaggtagaatt

SEQ ID NO: 105 - DNA, 21 bp, synthetic construct
  source 1..21: mol_type = other DNA
ttaaaatcctcttccctcctc

SEQ ID NO: 106 - DNA, 30 bp, synthetic construct
  source 1..30: mol_type = other DNA
atatgtgaaaaatagagttgataagtaagg

SEQ ID NO: 107 - DNA, 22 bp, synthetic construct
  source 1..22: mol_type = other DNA
cttaaaatcctcttccctcctc

SEQ ID NO: 108 - DNA, 15 bp, synthetic construct
  source 1..15: mol_type = other DNA
gatggtgcgagcgtc

SEQ ID NO: 109 - DNA, 23 bp, synthetic construct
  source 1..23: mol_type = other DNA
ctatctaaacctcaaaccaatcg

SEQ ID NO: 110 - DNA, 15 bp, synthetic construct
  source 1..15: mol_type = other DNA
tacaccgccccctcc

SEQ ID NO: 111 - DNA, 16 bp, synthetic construct
  source 1..16: mol_type = other DNA
tccgccgaccaatcac

SEQ ID NO: 112 - DNA, 18 bp, synthetic construct
  source 1..18: mol_type = other DNA
ccgaactcgaacgacaac

SEQ ID NO: 113 - DNA, 32 bp, synthetic construct
  source 1..32: mol_type = other DNA
ayggtaattttaagggtggatggtgygagygt

SEQ ID NO: 114 - DNA, 30 bp, synthetic construct
  source 1..30: mol_type = other DNA
crccccctccrccraccaatcacraaaact

SEQ ID NO: 115 - DNA, 43 bp, synthetic construct
  source 1..43: mol_type = other DNA
aagtaaggagatttaaggtagaattygaggtttayggagtagt

SEQ ID NO: 116 - DNA, 39 bp, synthetic construct
  source 1..39: mol_type = other DNA
accataacrcttaaaatcctcttccctcctcraatcrct

SEQ ID NO: 117 - DNA, 29 bp, synthetic construct
  source 1..29: mol_type = other DNA
ggagatttaaggtagaattcgaggtttac

SEQ ID NO: 118 - DNA, 22 bp, synthetic construct
  source 1..22: mol_type = other DNA
ctcgaacgacaacgaccataac

SEQ ID NO: 119 - DNA, 23 bp, synthetic construct
  source 1..23: mol_type = other DNA
gaattcgaggtttacggagtagt

SEQ ID NO: 120 - DNA, 19 bp, synthetic construct
  source 1..19: mol_type = other DNA
ctcctcgaatcgctacacc

SEQ ID NO: 121 - DNA, 22 bp, synthetic construct
  source 1..22: mol_type = other DNA
tttaagggtggatggtgcgagc

SEQ ID NO: 122 - DNA, 19 bp, synthetic construct
  source 1..19: mol_type = other DNA
ctcaacaaatacgcgaccc

SEQ ID NO: 123 - DNA, 22 bp, synthetic construct
  source 1..22: mol_type = other DNA
cggttaattacggaggttgttc

SEQ ID NO: 124 - DNA, 25 bp, synthetic construct
  source 1..25: mol_type = other DNA
cctacgaaacaattaccttctacga

SEQ ID NO: 125 - DNA, 21 bp, synthetic construct
  source 1..21: mol_type = other DNA
aaaacaaaacccgaaacctac

SEQ ID NO: 126 - DNA, 23 bp, synthetic construct
  source 1..23: mol_type = other DNA
tagtaagtacgcgattcgggttc

SEQ ID NO: 127 - DNA, 27 bp, synthetic construct
  source 1..27: mol_type = other DNA
gaaacctacgaaacaattaccttctac

SEQ ID NO: 128 - DNA, 21 bp, synthetic construct
  source 1..21: mol_type = other DNA
cggagtagttattttttacgg

SEQ ID NO: 129 - DNA, 18 bp, synthetic construct
  source 1..18: mol_type = other DNA
aacgacaacgaccataac

SEQ ID NO: 130 - DNA, 24 bp, synthetic construct
  source 1..24: mol_type = other DNA
gttacaattacctcaacaaatacg

SEQ ID NO: 131 - DNA, 20 bp, synthetic construct
  source 1..20: mol_type = other DNA
ggtagaattcgaggtttacg

SEQ ID NO: 132 - DNA, 18 bp, synthetic construct
  source 1..18: mol_type = other DNA
tcttccctcctcgaatcg

SEQ ID NO: 133 - DNA, 19 bp, synthetic construct
  source 1..19: mol_type = other DNA
caatcacgaaaactacccg

SEQ ID NO: 134 - DNA, 17 bp, synthetic construct
  source 1..17: mol_type = other DNA
gaactcgaacgacaacg

SEQ ID NO: 135 - DNA, 18 bp, synthetic construct
  source 1..18: mol_type = other DNA
aactcgaacgacaacgac

SEQ ID NO: 136 - DNA, 25 bp, synthetic construct
  source 1..25: mol_type = other DNA
cgttacaattacctcaacaaatacg

SEQ ID NO: 137 - DNA, 22 bp, synthetic construct
  source 1..22: mol_type = other DNA
ttaaaatcctcttccctcctcg

SEQ ID NO: 138 - DNA, 17 bp, synthetic construct
  source 1..17: mol_type = other DNA
atcctcttccctcctcg

SEQ ID NO: 139 - DNA, 21 bp, synthetic construct
  source 1..21: mol_type = other DNA
aggtagaattcgaggtttacg

SEQ ID NO: 140 - DNA, 15 bp, synthetic construct
  source 1..15: mol_type = other DNA
tacccacccgcttcg

SEQ ID NO: 141 - DNA, 22 bp, synthetic construct
  source 1..22: mol_type = other DNA
tgggaaaatggttttgagttcg

SEQ ID NO: 142 - DNA, 21 bp, synthetic construct
  source 1..21: mol_type = other DNA
gagggaagaggattttaagcg

SEQ ID NO: 143 - DNA, 24 bp, synthetic construct
  source 1..24: mol_type = other DNA
ccaaaacgatatccaaattctccg

SEQ ID NO: 144 - DNA, 19 bp, synthetic construct
  source 1..19: mol_type = other DNA
ggatcgtagggtgtttacg

SEQ ID NO: 145 - DNA, 23 bp, synthetic construct
  source 1..23: mol_type = other DNA
ctacgccctaaaaaactacatcg

SEQ ID NO: 146 - DNA, 23 bp, synthetic construct
  source 1..23: mol_type = other DNA
gaattcggagaatttggatatcg

SEQ ID NO: 147 - DNA, 21 bp, synthetic construct
  source 1..21: mol_type = other DNA
aactctccactacctactacg

SEQ ID NO: 148 - DNA, 26 bp, synthetic construct
  source 1..26: mol_type = other DNA
gcgtatttgttgaggtaattgtaacg

SEQ ID NO: 149 - DNA, 22 bp, synthetic construct
  source 1..22: mol_type = other DNA
actctataacctcgctattccg

SEQ ID NO: 150 - DNA, 23 bp, synthetic construct
  source 1..23: mol_type = other DNA
aggagggaagaggattttaagcg

SEQ ID NO: 151 - DNA, 25 bp, synthetic construct
  source 1..25: mol_type = other DNA
cccaaaacgatatccaaattctccg

SEQ ID NO: 152 - DNA, 21 bp, synthetic construct
  source 1..21: mol_type = other DNA
ggggatcgtagggtgtttacg

SEQ ID NO: 153 - DNA, 27 bp, synthetic construct
  source 1..27: mol_type = other DNA
ctcactacgccctaaaaaactacatcg

SEQ ID NO: 154 - DNA, 24 bp, synthetic construct
  source 1..24: mol_type = other DNA
tcggttaattacggaggttgttcg

SEQ ID NO: 155 - DNA, 26 bp, synthetic construct
  source 1..26: mol_type = other DNA
aacctacgaaacaattaccttctacg

SEQ ID NO: 156 - DNA, 28 bp, synthetic construct
  source 1..28: mol_type = other DNA
gagtttagggcggtatttaaatttttcg

SEQ ID NO: 157 - DNA, 21 bp, synthetic construct
  source 1..21: mol_type = other DNA
aaactccaaacgccataaccg

SEQ ID NO: 158 - DNA, 22 bp, synthetic construct
  source 1..22: mol_type = other DNA
ttaagcgttatggtcgttgtcg

SEQ ID NO: 159 - DNA, 21 bp, synthetic construct
  source 1..21: mol_type = other DNA
gcgcgataaaaacccaaaacg

SEQ ID NO: 160 - DNA, 31 bp, synthetic construct
  source 1..31: mol_type = other DNA
acacgacaacgtctataaatatcgccgaacc

SEQ ID NO: 161 - DNA, 28 bp, synthetic construct
  source 1..28: mol_type = other DNA
cccgacgatactcataaacgctaccgta

SEQ ID NO: 162 - DNA, 26 bp, synthetic construct
  source 1..26: mol_type = other DNA
ccgtaactacgtccccaaaaccgaaa

SEQ ID NO: 163 - DNA, 24 bp, synthetic construct
  source 1..24: mol_type = other DNA
tcgggtttaggaggtcgtgtgagg

SEQ ID NO: 164 - DNA, 24 bp, synthetic construct
  source 1..24: mol_type = other DNA
aaccgtataaaaatcccgcaataa

SEQ ID NO: 165 - DNA, 28 bp, synthetic construct
  source 1..28: mol_type = other DNA
aaacgcaactacgacgcctaattcgtac

SEQ ID NO: 166 - DNA, 27 bp, synthetic construct
  source 1..27: mol_type = other DNA
ttggcgcgtatagatacgattcggagt

SEQ ID NO: 167 - DNA, 22 bp, synthetic construct
  source 1..22: mol_type = other DNA
tagtgcgtttgtagtttcgagt

SEQ ID NO: 168 - DNA, 21 bp, synthetic construct
  source 1..21: mol_type = other DNA
ctcccgattctaaaaacgcaa

SEQ ID NO: 169 - DNA, 17 bp, synthetic construct
  source 1..17: mol_type = other DNA
acgtagttacggcgttt

SEQ ID NO: 170 - DNA, 19 bp, synthetic construct
  source 1..19: mol_type = other DNA
caacgaccaaataccctca

SEQ ID NO: 171 - DNA, 22 bp, synthetic construct
  source 1..22: mol_type = other DNA
ttcgcgtcgttcgttatcgttt

SEQ ID NO: 172 - DNA, 22 bp, synthetic construct
  source 1..22: mol_type = other DNA
agcgtggttcgagtttcggttt

SEQ ID NO: 173 - DNA, 23 bp, synthetic construct
  source 1..23: mol_type = other DNA
atttggtcgttgcgttgggttgg

SEQ ID NO: 174 - DNA, 19 bp, synthetic construct
  source 1..19: mol_type = other DNA
cccgccaccgtctcgtaat

SEQ ID NO: 175 - DNA, 20 bp, synthetic construct
  source 1..20: mol_type = other DNA
ttgcgagggcgaggacgagg

SEQ ID NO: 176 - DNA, 26 bp, synthetic construct
  source 1..26: mol_type = other DNA
cgaggacgagggtaaagatttagcgt

SEQ ID NO: 177 - DNA, 32 bp, synthetic construct
  source 1..32: mol_type = other DNA
aacgcaacgatatacacaaccacataaccaac

SEQ ID NO: 178 - DNA, 29 bp, synthetic construct
  source 1..29: mol_type = other DNA
ttcgagtttcggtttttattcggtcgtgt

SEQ ID NO: 179 - DNA, 21 bp, synthetic construct
  source 1..21: mol_type = other DNA
ttcggtttttattcggtcgtg

SEQ ID NO: 180 - DNA, 29 bp, synthetic construct
  source 1..29: mol_type = other DNA
caccgaccctaaaatcctaaaaaaccgat

SEQ ID NO: 181 - DNA, 26 bp, synthetic construct
  source 1..26: mol_type = other DNA
accgataaacgacgtacgcgaaaact

SEQ ID NO: 182 - DNA, 27 bp, synthetic construct
  source 1..27: mol_type = other DNA
ctacgaaacgataacgaacgacgcgaa

SEQ ID NO: 183 - DNA, 21 bp, synthetic construct
  source 1..21: mol_type = other DNA
acgagggtaaagatttagcgt

SEQ ID NO: 184 - DNA, 22 bp, synthetic construct
  source 1..22: mol_type = other DNA
cacaccgctacgcccgtaccaa

SEQ ID NO: 185 - DNA, 18 bp, synthetic construct
  source 1..18: mol_type = other DNA
tgagcggcgtgcgcggag

SEQ ID NO: 186 - DNA, 21 bp, synthetic construct
  source 1..21: mol_type = other DNA
agtttagagagattaggggcg

SEQ ID NO: 187 - DNA, 25 bp, synthetic construct
  source 1..25: mol_type = other DNA
tacgcgattccccaaccctcgcgac

SEQ ID NO: 188 - DNA, 20 bp, synthetic construct
  source 1..20: mol_type = other DNA
aaggcgcggcgttcggttag

SEQ ID NO: 189 - DNA, 26 bp, synthetic construct
  source 1..26: mol_type = other DNA
tcaaaaccattttcccacgaaataaa

SEQ ID NO: 190 - DNA, 24 bp, synthetic construct
  source 1..24: mol_type = other DNA
ctctataacctcgctattccgcct

SEQ ID NO: 191 - DNA, 28 bp, synthetic construct
  source 1..28: mol_type = other DNA
cccacgaaataaaaaccaaaacgccaac

SEQ ID NO: 192 - DNA, 23 bp, synthetic construct
  source 1..23: mol_type = other DNA
actcaaaaccattttcccacgaa

SEQ ID NO: 193 - DNA, 25 bp, synthetic construct
  source 1..25: mol_type = other DNA
actcaaaaccattttcccacgaaat

SEQ ID NO: 194 - DNA, 27 bp, synthetic construct
  source 1..27: mol_type = other DNA
aacgaaaaacgccactacccgatacga

SEQ ID NO: 195 - DNA, 28 bp, synthetic construct
  source 1..28: mol_type = other DNA
aacgccactacccgatacgaactacacc

SEQ ID NO: 196 - DNA, 25 bp, synthetic construct
  source 1..25: mol_type = other DNA
aaaaaccaaaacgccaactacccca

SEQ ID NO: 197 - DNA, 24 bp, synthetic construct
  source 1..24: mol_type = other DNA
caaaacgccaactaccccaacgac

SEQ ID NO: 198 - DNA, 19 bp, synthetic construct
  source 1..19: mol_type = other DNA
tgcgagcgtcgttggggta

SEQ ID NO: 199 - DNA, 23 bp, synthetic construct
  source 1..23: mol_type = other DNA
tggtcgttgtcgttcgagttcgg

SEQ ID NO: 200 - DNA, 22 bp, synthetic construct
  source 1..22: mol_type = other DNA
cctcgctattccgcctaacgcg

SEQ ID NO: 201 - DNA, 24 bp, synthetic construct
  source 1..24: mol_type = other DNA
actacgcaaaatctaaacgaatca

SEQ ID NO: 202 - DNA, 22 bp, synthetic construct
  source 1..22: mol_type = other DNA
tatggtcgttgtcgttcgagtt

SEQ ID NO: 203 - DNA, 22 bp, synthetic construct
  source 1..22: mol_type = other DNA
tacgtaaacaccctacgatccc

SEQ ID NO: 204 - DNA, 20 bp, synthetic construct
  source 1..20: mol_type = other DNA
ttcgtttagattttgcgtag

SEQ ID NO: 205 - DNA, 23 bp, synthetic construct
  source 1..23: mol_type = other DNA
aacgatatccaaattctccgaat

SEQ ID NO: 206 - DNA, 23 bp, synthetic construct
  source 1..23: mol_type = other DNA
ttcgtttttcggtcgcgtttgtt

SEQ ID NO: 207 - DNA, 31 bp, synthetic construct
  source 1..31: mol_type = other DNA
atacgaacgccgctaaaacaactaacgttct

SEQ ID NO: 208 - DNA, 24 bp, synthetic construct
  source 1..24: mol_type = other DNA
taccgcccgaacccgaatcgcgta

SEQ ID NO: 209 - DNA, 19 bp, synthetic construct
  source 1..19: mol_type = other DNA
aagcggagaagattgcgta

SEQ ID NO: 210 - DNA, 23 bp, synthetic construct
  source 1..23: mol_type = other DNA
tttaggagtgagtggaagataga

SEQ ID NO: 211 - DNA, 23 bp, synthetic construct
  source 1..23: mol_type = other DNA
aaaccacaccatcctaattacct

SEQ ID NO: 212 - DNA, 23 bp, synthetic construct
  source 1..23: mol_type = other DNA
cccaaaacacatttcttccattc